European Patent Specification EP 3 904 376 B1, published November 13, 2024. Title: Mutant Factor VIII Compositions and Methods. Applicant: Xiao, Weidong. The sequence listing filed with the application follows.

SEQUENCE LISTING (9 sequences)

SEQ ID NO: 1 - DNA, 7056 bp, Homo sapiens
atgcaaatagagctctccacctgcttctttctgtgccttttgcgattctgctttagtgccaccagaagatactacctgggtgcagtggaactgtcatgggactatatgcaaagtgatctcggtgagctgcctgtggacgcaagatttcctcctagagtgccaaaatcttttccattcaacacctcagtcgtgtacaaaaagactctgtttgtagaattcacggatcaccttttcaacatcgctaagccaaggccaccctggatgggtctgctaggtcctaccatccaggctgaggtttatgatacagtggtcattacacttaagaacatggcttcccatcctgtcagtcttcatgctgttggtgtatcctactggaaagcttctgagggagctgaatatgatgatcagaccagtcaaagggagaaagaagatgataaagtcttccctggtggaagccatacatatgtctggcaggtcctgaaagagaatggtccaatggcctctgacccactgtgccttacctactcatatctttctcatgtggacctggtaaaagacttgaattcaggcctcattggagccctactagtatgtagagaagggagtctggccaaggaaaagacacagaccttgcacaaatttatactactttttgctgtatttgatgaagggaaaagttggcactcagaaacaaagaactccttgatgcaggatagggatgctgcatctgctcgggcctggcctaaaatgcacacagtcaatggttatgtaaacaggtctctgccaggtctgattggatgccacaggaaatcagtctattggcatgtgattggaatgggcaccactcctgaagtgcactcaatattcctcgaaggtcacacatttcttgtgaggaaccatcgccaggcgtccttggaaatctcgccaataactttccttactgctcaaacactcttgatggaccttggacagtttctactgttttgtcatatctcttcccaccaacatgatggcatggaagcttatgtcaaagtagacagctgtccagaggaaccccaactacgaatgaaaaataatgaagaagcggaagactatgatgatgatcttactgattctgaaatggatgtggtcaggtttgatgatgacaactctccttcctttatccaaattcgctcagttgccaagaagcatcctaaaacttgggtacattacattgctgctgaagaggaggactgggactatgctcccttagtcctcgcccccgatgacagaagttataaaagtcaatatttgaacaatggccctcagcggattggtaggaagtacaaaaaagtccgatttatggcatacacagatgaaacctttaagactcgtgaagctattcagcatgaatcaggaatcttgggacctttactttatggggaagttggagacacactgttgattatatttaagaatcaagcaagcagaccatataacatctaccctcacggaatcactgatgtccgtcctttgtattcaaggagattaccaaaaggtgtaaaacatttgaaggattttccaattctgccaggagaaatattcaaatataaatggacagtgactgtagaagatgggccaactaaatcagatcctcggtgcctgacccgctattactctagtttcgttaatatggagagagatctagcttcaggactcattggccctctcctcatctgctacaaagaatctgtagatcaaagaggaaaccagataatgtcagacaagaggaatgtcatcctgttttctgtatttgatgagaaccgaagctggtacctcacagagaatatacaacgctttctccccaatccagctggagtgcagcttgaggatccagagttccaagcctccaacatcatgcacagcatcaatggctatgtttttgatagtttgcagttgtcagtttgtttgcatgaggtggcatactggtacattctaagcattggagcacagactgacttcctttctgtcttcttctctggatataccttcaaacacaaaatggtctatgaagacacactcaccctattcccattctcaggagaaactgtcttcatgtcgatggaaaacccaggtctatggattctggggtgccacaactcagactttcggaacagaggcatgaccgccttactgaaggtttctagttgtgacaagaacactggtgattattacgaggacagttatgaagatatttcagcatacttgctgagtaaaaacaatgccattgaaccaagaagcttctcccagaattcaagacaccgtagcactaggcaaaagcaatttaatgccaccacaattccagaaaatgacatagagaagactgacccttggtttgcacacagaacacctatgcctaaaatacaaaatgtctcctctagtgatttgttgatgctcttgcgacagagtcctactccacatgggctatccttatctgatctccaagaagccaaatatgagactttttctgatgatccatcacctggagcaatagacagtaataacagcctgtctgaaatgacacacttcaggccacagctccatcacagtggggacatggtatttacccctgagtcaggcctccaattaagattaaatgagaaactggggacaactgcagcaacagagttgaagaaacttgatttcaaagtttctagtacatcaaataatctgatttcaacaattccatcagacaatttggcagcaggtactgataatacaagttccttaggacccccaagtatgccagttcattatgatagtcaattagataccactctatttggcaaaaagtcatctccccttactgagtctggtggacctctgagcttgagtgaagaaaataatgattcaaagttgttagaatcaggtttaatgaatagccaagaaagttcatggggaaaaaatgtatcgtcaacagagagtggtaggttatttaaagggaaaagagctcatggacctgctttgttgactaaagataatgccttattcaaagttagcatctctttgttaaagacaaacaaaacttccaataattcagcaactaatagaaagactcacattgatggcccatcattattaattgagaatagtccatcagtctggcaaaatatattagaaagtgacactgagtttaaaaaagtgacacctttgattcatgacagaatgcttatggacaaaaatgctacagctttgaggctaaatcatatgtcaaataaaactacttcatcaaaaaacatggaaatggtccaacagaaaaaagagggccccattccaccagatgcacaaaatccagatatgtcgttctttaagatgctattcttgccagaatcagcaaggtggatacaaaggactcatggaaagaactctctgaactctgggcaaggccccagtccaaagcaattagtatccttaggaccagaaaaatctgtggaaggtcagaatttcttgtctgagaaaaacaaagtggtagtaggaaagggtgaatttacaaaggacgtaggactcaaagagatggtttttccaagcagcagaaacctatttcttactaacttggataatttacatgaaaataatacacacaatcaagaaaaaaaaattcaggaagaaatagaaaagaaggaaacattaatccaagagaatgtagttttgcctcagatacatacagtgactggcactaagaatttcatgaagaaccttttcttactgagcactaggcaaaatgtagaaggttcatatgacggggcatatgctccagtacttcaagattttaggtcattaaatgattcaacaaatagaacaaagaaacacacagctcatttctcaaaaaaaggggaggaagaaaacttggaaggcttgggaaatcaaaccaagcaaattgtagagaaatatgcatgcaccacaaggatatctcctaatacaagccagcagaattttgtcacgcaacgtagtaagagagctttgaaacaattcagactcccactagaagaaacagaacttgaaaaaaggataattgtggatgacacctcaacccagtggtccaaaaacatgaaacatttgaccccgagcaccctcacacagatagactacaatgagaaggagaaaggggccattactcagtctcccttatcagattgccttacgaggagtcatagcatccctcaagcaaatagatctccattacccattgcaaaggtatcatcatttccatctattagacctatatatctgaccagggtcctattccaagacaactcttctcatcttccagcagcatcttatagaaagaaagattctggggtccaagaaagcagtcatttcttacaaggagccaaaaaaaataacctttctttagccattctaaccttggagatgactggtgatcaaagagaggttggctccctggggacaagtgccacaaattcagtcacatacaagaaagttgagaacactgttctcccgaaaccagacttgcccaaaacatctggcaaagttgaattgcttccaaaagttcacatttatcagaaggacctattccctacggaaactagcaatgggtctcctggccatctggatctcgtggaagggagccttcttcagggaacagagggagcgattaagtggaatgaagcaaacagacctggaaaagttccctttctgagagtagcaacagaaagctctgcaaagactccctccaagctattggatcctcttgcttgggataaccactatggtactcagataccaaaagaagagtggaaatcccaagagaagtcaccagaaaaaacagcttttaagaaaaaggataccattttgtccctgaacgcttgtgaaagcaatcatgcaatagcagcaataaatgagggacaaaataagcccgaaatagaagtcacctgggcaaagcaaggtaggactgaaaggctgtgctctcaaaacccaccagtcttgaaacgccatcaacgggaaataactcgtactactcttcagtcagatcaagaggaaattgactatgatgataccatatcagttgaaatgaagaaggaagattttgacatttatgatgaggatgaaaatcagagcccccgcagctttcaaaagaaaacacgacactattttattgctgcagtggagaggctctgggattatgggatgagtagctccccacatgttctaagaaacagggctcagagtggcagtgtccctcagttcaagaaagttgttttccaggaatttactgatggctcctttactcagcccttataccgtggagaactaaatgaacatttgggactcctggggccatatataagagcagaagttgaagataatatcatggtaactttcagaaatcaggcctctcgtccctattccttctattctagccttatttcttatgaggaagatcagaggcaaggagcagaacctagaaaaaactttgtcaagcctaatgaaaccaaaacttacttttggaaagtgcaacatcatatggcacccactaaagatgagtttgactgcaaagcctgggcttatttctctgatgttgacctggaaaaagatgtgcactcaggcctgattggaccccttctggtctgccacactaacacactgaaccctgctcatgggagacaagtgacagtacaggaatttgctctgtttttcaccatctttgatgagaccaaaagctggtacttcactgaaaatatggaaagaaactgcagggctccctgcaatatccagatggaagatcccacttttaaagagaattatcgcttccatgcaatcaatggctacataatggatacactacctggcttagtaatggctcaggatcaaaggattcgatggtatctgctcagcatgggcagcaatgaaaacatccattctattcatttcagtggacatgtgttcactgtacgaaaaaaagaggagtataaaatggcactgtacaatctctatccaggtgtttttgagacagtggaaatgttaccatccaaagctggaatttggcgggtggaatgccttattggcgagcatctacatgctgggatgagcacactttttctggtgtacagcaataagtgtcagactcccctgggaatggcttctggacacattagagattttcagattacagcttcaggacaatatggacagtgggccccaaagctggccagacttcattattccggatcaatcaatgcctggagcaccaaggagcccttttcttggatcaaggtggatctgttggcaccaatgattattcacggcatcaagacccagggtgcccgtcagaagttctccagcctctacatctctcagtttatcatcatgtatagtcttgatgggaagaagtggcagacttatcgaggaaattccactggaaccttaatggtcttctttggcaatgtggattcatctgggataaaacacaatatttttaaccctccaattattgctcgatacatccgtttgcacccaactcattatagcattcgcagcactcttcgcatggagttgatgggctgtgatttaaatagttgcagcatgccattgggaatggagagtaaagcaatatcagatgcacagattactgcttcatcctactttaccaatatgtttgccacctggtctccttcaaaagctcgacttcacctccaagggaggagtaatgcctggagacctcaggtgaataatccaaaagagtggctgcaagtggacttccagaagacaatgaaagtcacaggagtaactactcagggagtaaaatctctgcttaccagcatgtatgtgaaggagttcctcatctccagcagtcaagatggccatcagtggactctcttttttcagaatggcaaagtaaaggtttttcagggaaatcaagactccttcacacctgtggtgaactctctagacccaccgttactgactcgctaccttcgaattcacccccagagttgggtgcaccagattgccctgaggatggaggttctgggctgcgaggcacaggacctctactga

SEQ ID NO: 2 - protein, 2332 aa, Homo sapiens
ATRRYYLGAVELSWDYMQSDLGELPVDARFPPRVPKSFPFNTSVVYKKTLFVEFTDHLFNIAKPRPPWMGLLGPTIQAEVYDTVVITLKNMASHPVSLHAVGVSYWKASEGAEYDDQTSQREKEDDKVFPGGSHTYVWQVLKENGPMASDPLCLTYSYLSHVDLVKDLNSGLIGALLVCREGSLAKEKTQTLHKFILLFAVFDEGKSWHSETKNSLMQDRDAASARAWPKMHTVNGYVNRSLPGLIGCHRKSVYWHVIGMGTTPEVHSIFLEGHTFLVRNHRQASLEISPITFLTAQTLLMDLGQFLLFCHISSHQHDGMEAYVKVDSCPEEPQLRMKNNEEAEDYDDDLTDSEMDVVRFDDDNSPSFIQIRSVAKKHPKTWVHYIAAEEEDWDYAPLVLAPDDRSYKSQYLNNGPQRIGRKYKKVRFMAYTDETFKTREAIQHESGILGPLLYGEVGDTLLIIFKNQASRPYNIYPHGITDVRPLYSRRLPKGVKHLKDFPILPGEIFKYKWTVTVEDGPTKSDPRCLTRYYSSFVNMERDLASGLIGPLLICYKESVDQRGNQIMSDKRNVILFSVFDENRSWYLTENIQRFLPNPAGVQLEDPEFQASNIMHSINGYVFDSLQLSVCLHEVAYWYILSIGAQTDFLSVFFSGYTFKHKMVYEDTLTLFPFSGETVFMSMENPGLWILGCHNSDFRNRGMTALLKVSSCDKNTGDYYEDSYEDISAYLLSKNNAIEPRSFSQNSRHPSTRQKQFNATTIPENDIEKTDPWFAHRTPMPKIQNVSSSDLLMLLRQSPTPHGLSLSDLQEAKYETFSDDPSPGAIDSNNSLSEMTHFRPQLHHSGDMVFTPESGLQLRLNEKLGTTAATELKKLDFKVSSTSNNLISTIPSDNLAAGTDNTSSLGPPSMPVHYDSQLDTTLFGKKSSPLTESGGPLSLSEENNDSKLLESGLMNSQESSWGKNVSSTESGRLFKGKRAHGPALLTKDNALFKVSISLLKTNKTSNNSATNRKTHIDGPSLLIENSPSVWQNILESDTEFKKVTPLIHDRMLMDKNATALRLNHMSNKTTSSKNMEMVQQKKEGPIPPDAQNPDMSFFKMLFLPESARWIQRTHGKNSLNSGQGPSPKQLVSLGPEKSVEGQNFLSEKNKVVVGKGEFTKDVGLKEMVFPSSRNLFLTNLDNLHENNTHNQEKKIQEEIEKKETLIQENVVLPQIHTVTGTKNFMKNLFLLSTRQNVEGSYDGAYAPVLQDFRSLNDSTNRTKKHTAHFSKKGEEENLEGLGNQTKQIVEKYACTTRISPNTSQQNFVTQRSKRALKQFRLPLEETELEKRIIVDDTSTQWSKNMKHLTPSTLTQIDYNEKEKGAITQSPLSDCLTRSHSIPQANRSPLPIAKVSSFPSIRPIYLTRVLFQDNSSHLPAASYRKKDSGVQESSHFLQGAKKNNLSLAILTLEMTGDQREVGSLGTSATNSVTYKKVENTVLPKPDLPKTSGKVELLPKVHIYQKDLFPTETSNGSPGHLDLVEGSLLQGTEGAIKWNEANRPGKVPFLRVATESSAKTPSKLLDPLAWDNHYGTQIPKEEWKSQEKSPEKTAFKKKDTILSLNACESNHAIAAINEGQNKPEIEVTWAKQGRTERLCSQNPPVLKRHQREITRTTLQSDQEEIDYDDTISVEMKKEDFDIYDEDENQSPRSFQKKTRHYFIAAVERLWDYGMSSSPHVLRNRAQSGSVPQFKKVVFQEFTDGSFTQPLYRGELNEHLGLLGPYIRAEVEDNIMVTFRNQASRPYSFYSSLISYEEDQRQGAEPRKNFVKPNETKTYFWKVQHHMAPTKDEFDCKAWAYFSDVDLEKDVHSGLIGPLLVCHTNTLNPAHGRQVTVQEFALFFTIFDETKSWYFTENMERNCRAPCNIQMEDPTFKENYRFHAINGYIMDTLPGLVMAQDQRIRWYLLSMGSNENIHSIHFSGHVFTVRKKEEYKMALYNLYPGVFETVEMLPSKAGIWRVECLIGEHLHAGMSTLFLVYSNKCQTPLGMASGHIRDFQITASGQYGQWAPKLARLHYSGSINAWSTKEPFSWIKVDLLAPMIIHGIKTQGARQKFSSLYISQFIIMYSLDGKKWQTYRGNSTGTLMVFFGNVDSSGIKHNIFNPPIIARYIRLHPTHYSIRSTLRMELMGCDLNSCSMPLGMESKAISDAQITASSYFTNMFATWSPSKARLHLQGRSNAWRPQVNNPKEWLQVDFQKTMKVTGVTTQGVKSLLTSMYVKEFLISSSQDGHQWTLFFQNGKVKVFQGNQDSFTPVVNSLDPPLLTRYLRIHPQSWVHQIALRMEVLGCEAQDLY

SEQ ID NO: 3 - DNA, 9720 bp, Artificial Sequence
  pAAV-CB-hBDD-F8-X10
aattcccatcatcaataatataccttattttggattgaagccaatatgataatgagggggtggagtttgtgacgtggcgcggggcgtgggaacggggcgggtgacgtagtagtctctagaggtccccagcgaccttgacgggcatctgcccggcatttctgacagctttgtgaactgggtggccgagaaggaatgggagttgccgccagattctgacatggatctgaatctgattgagcaggcacccctgaccgtggccgagaagctgcatcgctggcgtaatagcgaagaggcccgcaccgatcgcccttcccaacagttgcgcagcctgaatggcgaatggaattccagacgattgagcgtcaaaatgtaggtatttccatgagcgtttttcctgttgcaatggctggcggtaatattgttctggatattaccagcaaggccgatagtttgagttcttctactcaggcaagtgatgttattactaatcaaagaagtattgcgacaacggttaatttgcgtgatggacagactcttttactcggtggcctcactgattataaaaacacttctcaggattctggcgtaccgttcctgtctaaaatccctttaatcggcctcctgtttagctcccgctctgattctaacgaggaaagcacgttatacgtgctcgtcaaagcaaccatagtacgcgccctgtagcggcgcattaagcgcggcgggtgtggtggttacgcgcagcgtgaccgctacacttgccagcgccctagcgcccgctcctttcgctttcttcccttcctttctcgccacgttcgccggctttccccgtcaagctctaaatcgggggctccctttagggttccgatttagtgctttacggcacctcgaccccaaaaaacttgattagggtgatggttcacgtagtgggccatcgccctgatagacggtttttcgccctttgacgttggagtccacgttctttaatagtggactcttgttccaaactggaacaacactcaaccctatctcggtctattcttttgatttataagggattttgccgatttcggcctattggttaaaaaatgagctgatttaacaaaaatttaacgcgaattttaacaaaatattaacgtttacaatttaaatatttgcttatacaatcttcctgtttttggggcttttctgattatcaaccggggtacatatgattgacatgctagttttacgattaccgttcatcgcctgcaggggggggggggggggggttggccactccctctctgcgcgctcgctcgctcactgaggccgggcgaccaaaggtcgcccgacgcccgggctttgcccgggcggcctcagtgagcgagcgagcgcgcagagagggagtggccaactccatcactaggggttcctagatctgaattcggtacgtacctctggtcgttacataacttacggtaaatggcccgcctggctgaccgcccaacgaccccgcccattgacgtcaataatgacgtatgttcccatagtaacgccaatagggactttccattgacgtcaatgggtggagtatttacggtaaactgcccacttggcagtacatcaagtgtatcatatgccaagtacgccccctattgacgtcaatgacggtaaatggcccgcctggcattatgcccagtacatgaccttatgggactttcctacttggcagtacatctactcgaggccacgttctgcttcactctccccatctcccccccctccccacccccaattttgtatttatttattttttaattattttgtgcagcgatgggggcggggggggggggggggggggcgcgcgccaggcggggcggggcggggcgaggggcggggcggggcgaggcggagaggtgcggcggcagccaatcagagcggcgcgctccgaaagtttccttttatggcgaggcggcggcggcggcggccctataaaaagcgaagcgcgcggcgggcgggagcgggatcagccaccgcggtggcggcctagagtcgacgaggaactgaaaaaccagaaagttaactggtaagtttagtctttttgtcttttatttcaggtcccggatccggtggtggtgcaaatcaaagaactgctcctcagtggatgttgcctttacttctaggcctgtacggaagtgttacttctgctctaaaagctgcggaattgtacccgcggccgcttttcaaaatgcaaatagagctctccacctgcttctttctgtgccttttgcgattctgctttagtgccaccagaagatactacctgggtgcagtggaactgtcatgggactatatgcaaagtgatctcggtgagctgcctgtggacgcaagatttcctcctagagtgccaaaatcttttccattcaacacctcagtcgtgtacaaaaagactctgtttgtagaattcacggatcaccttttcaacatcgctaagccaaggccaccctggatgggtctgctaggtcctaccatccaggctgaggtttacgacacggtggtcgttaccctgaagaacatggcttctcatcccgttagtcttcacgctgtcggcgtctccttctggaaatcttccgaaggcgctgaatatgaggatcacaccagccaaagggagaaggaagacgataaagtccttcccggtaaaagccaaacctacgtctggcaggtcctgaaagaaaatggtccaacagcctctgacccaccatgtcttacctactcatacctgtctcacgtggacctggtgaaagacctgaattcgggcctcattggagccctactagtatgtagagaagggagtctggccaaggaaaagacacagaccttgcacaaatttatactactttttgctgtatttgatgaagggaaaagttggcactcagaaacaaagaactccttgatgcaggatagggatgctgcatctgctcgggcctggcctaaaatgcacacagtcaatggttatgtaaacaggtctctgccaggtctgattggatgccacaggaaatcagtctattggcatgtgattggaatgggcaccactcctgaagtgcactcaatattcctcgaaggtcacacatttcttgtgaggaaccatcgccaggcgtccttggaaatctcgccaataactttccttactgctcaaacactcttgatggaccttggacagtttctactgttttgtcatatctcttcccaccaacatgatggcatggaagcttatgtcaaagtagacagctgtccagaggaaccccaactacgaatgaaaaataatgaagaagcggaagactatgatgatgatcttactgattctgaaatggatgtggtcaggtttgatgatgacaactctccttcctttatccaaattcgctcagttgccaagaagcatcctaaaacttgggtacattacattgctgctgaagaggaggactgggactatgctcccttagtcctcgcccccgatgacagaagttataaaagtcaatatttgaacaatggccctcagcggattggtaggaagtacaaaaaagtccgatttatggcatacacagatgaaacctttaagactcgtgaagctattcagcatgaatcaggaatcttgggacctttactttatggggaagttggagacacactgttgattatatttaagaatcaagcaagcagaccatataacatctaccctcacggaatcactgatgtccgtcctttgtattcaaggagattaccaaaaggtgtaaaacatttgaaggattttccaattctgccaggagaaatattcaaatataaatggacagtgactgtagaagatgggccaactaaatcagatcctcggtgcctgacccgctattactctagtttcgttaatatggagagagatctagcttcaggactcattggccctctcctcatctgctacaaagaatctgtagatcaaagaggaaaccagataatgtcagacaagaggaatgtcatcctgttttctgtatttgatgagaaccgaagctggtacctcacagagaatatacaacgctttctccccaatccagctggagtgcagcttgaggatccagagttccaagcctccaacatcatgcacagcatcaatggctatgtttttgatagtttgcagttgtcagtttgtttgcatgaggtggcatactggtacattctaagcattggagcacagactgacttcctttctgtcttcttctctggatataccttcaaacacaaaatggtctatgaagacacactcaccctattcccattctcaggagaaactgtcttcatgtcgatggaaaacccaggtctatggattctggggtgccacaactcagactttcggaacagaggcatgaccgccttactgaaggtttctagttgtgacaagaacactggtgattattacgaggacagttatgaagatatttcagcatacttgctgagtaaaaacaatgccattgaaccaagaagcttctcccagaattcaagacaccctagcactaggcaaaagcaatttaatgccaccacaccaccagtcttgaaacgccatcaacgcgaaataactcgtactactcttcagtcagatcaagaggaaattgactatgatgataccatatcagttgaaatgaagaaggaagattttgacatttatgatgaggatgaaaatcagagcccccgcagctttcaaaagaaaacacgacactattttattgctgcagtggagaggctctgggattatgggatgagtagctccccacatgttctaagaaacagggctcagagtggcagtgtccctcagttcaagaaagttgttttccaggaatttactgatggctcctttactcagcccttataccgtggagaactaaatgaacatttgggactcctggggccatatataagagcagaagttgaagataatatcatggtaactttcagaaatcaggcctctcgtccctattccttctattctagccttatttcttatgaggaagatcagaggcaaggagcagaacctagaaaaaactttgtcaagcctaatgaaaccaaaacttacttttggaaagtgcaacatcatatggcacccactaaagatgagtttgactgcaaagcctgggcttatttctctgatgttgacctggaaaaagatgtgcactcaggcctgattggaccccttctggtctgccacactaacacactgaaccctgctcatgggagacaagtgacagtacaggaatttgctctgtttttcaccatctttgatgagaccaaaagctggtacttcactgaaaatatggaaagaaactgcagggctccctgcaatatccagatggaagatcccacttttaaagagaattatcgcttccatgcaatcaatggctacataatggatacactacctggcttagtaatggctcaggatcaaaggattcgatggtatctgctcagcatgggcagcaatgaaaacatccattctattcatttcagtggacatgtgttcactgtacgaaaaaaagaggagtataaaatggcactgtacaatctctatccaggtgtttttgagacagtggaaatgttaccatccaaagctggaatttggcgggtggaatgccttattggcgagcatctacatgctgggatgagcacactttttctggtgtacagcaataagtgtcagactcccctgggaatggcttctggacacattagagattttcagattacagcttcaggacaatatggacagtgggccccaaagctggccagacttcattattccggatcaatcaatgcctggagcaccaaggagcccttttcttggatcaaggtggatctgttggcaccaatgattattcacggcatcaagacccagggtgcccgtcagaagttctccagcctctacatctctcagtttatcatcatgtatagtcttgatgggaagaagtggcagacttatcgaggaaattccactggaaccttaatggtcttctttggcaatgtggattcatctgggataaaacacaatatttttaaccctccaattattgctcgatacatccgtttgcacccaactcattatagcattcgcagcactcttcgcatggagttgatgggctgtgatttaaatagttgcagcatgccattgggaatggagagtaaagcaatatcagatgcacagattactgcttcatcctactttaccaatatgtttgccacctggtctccttcaaaagctcgacttcacctccaagggaggagtaatgcctggagacctcaggtgaataatccaaaagagtggctgcaagtggacttccagaagacaatgaaagtcacaggagtaactactcagggagtaaaatctctgcttaccagcatgtatgtgaaggagttcctcatctccagcagtcaagatggccatcagtggactctcttttttcagaatggcaaagtaaaggtttttcagggaaatcaagactccttcacacctgtggtgaactctctagacccaccgttactgactcgctaccttcgaattcacccccagagttgggtgcaccagattgccctgaggatggaggttctgggctgcgaggcacaggacctctactgacaattgacgctgatcagcctcgactgtgccttctagttgccagccatctgttgtttgcccctcccccgtgccttccttgaccctggaaggtgccactcccactgtcctttcctaataaaatgaggaaattgcatcgcattgtctgagtaggtgtcattctattctggggggtggggtggggcaggacagcaagggggaggattgggaagacaatagcaggcatgctggggagagatctaggaacccctagtgatggagttggccactccctctctgcgcgctcgctcgctcactgaggccgcccgggcaaagcccgggcgtcgggcgacctttggtcgcccggcctcagtgagcgagcgagcgcgcagagagggagtggccaacccccccccccccccccctgcaggcgattctcttgtttgctccagactctcaggcaatgacctgatagcctttgtagagacctctcaaaaatagctaccctctccggcatgaatttatcagctagaacggttgaatatcatattgatggtgatttgactgtctccggcctttctcacccgtttgaatctttacctacacattactcaggcattgcatttaaaatatatgagggttctaaaaatttttatccttgcgttgaaataaaggcttctcccgcaaaagtattacagggtcataatgtttttggtacaaccgatttagctttatgctctgaggctttattgcttaattttgctaattctttgccttgcctgtatgatttattggatgttggaattcctgatgcggtattttctccttacgcatctgtgcggtatttcacaccgcatatggtgcactctcagtacaatctgctctgatgccgcatagttaagccagccccgacacccgccaacacccgctgacgcgccctgacgggcttgtctgctcccggcatccgcttacagacaagctgtgaccgtctccgggagctgcatgtgtcagaggttttcaccgtcatcaccgaaacgcgcgagacgaaagggcctcgtgatacgcctatttttataggttaatgtcatgataataatggtttcttagacgtcaggtggcacttttcggggaaatgtgcgcggaacccctatttgtttatttttctaaatacattcaaatatgtatccgctcatgagacaataaccctgataaatgcttcaataatattgaaaaaggaagagtatgagtattcaacatttccgtgtcgcccttattcccttttttgcggcattttgccttcctgtttttgctcacccagaaacgctggtgaaagtaaaagatgctgaagatcagttgggtgcacgagtgggttacatcgaactggatctcaacagcggtaagatccttgagagttttcgccccgaagaacgttttccaatgatgagcacttttaaagttctgctatgtggcgcggtattatcccgtattgacgccgggcaagagcaactcggtcgccgcatacactattctcagaatgacttggttgagtactcaccagtcacagaaaagcatcttacggatggcatgacagtaagagaattatgcagtgctgccataaccatgagtgataacactgcggccaacttacttctgacaacgatcggaggaccgaaggagctaaccgcttttttgcacaacatgggggatcatgtaactcgccttgatcgttgggaaccggagctgaatgaagccataccaaacgacgagcgtgacaccacgatgcctgtagcaatggcaacaacgttgcgcaaactattaactggcgaactacttactctagcttcccggcaacaattaatagactggatggaggcggataaagttgcaggaccacttctgcgctcggcccttccggctggctggtttattgctgataaatctggagccggtgagcgtgggtctcgcggtatcattgcagcactggggccagatggtaagccctcccgtatcgtagttatctacacgacggggagtcaggcaactatggatgaacgaaatagacagatcgctgagataggtgcctcactgattaagcattggtaactgtcagaccaagtttactcatatatactttagattgatttaaaacttcatttttaatttaaaaggatctaggtgaagatcctttttgataatctcatgaccaaaatcccttaacgtgagttttcgttccactgagcgtcagaccccgtagaaaagatcaaaggatcttcttgagatcctttttttctgcgcgtaatctgctgcttgcaaacaaaaaaaccaccgctaccagcggtggtttgtttgccggatcaagagctaccaactctttttccgaaggtaactggcttcagcagagcgcagataccaaatactgtccttctagtgtagccgtagttaggccaccacttcaagaactctgtagcaccgcctacatacctcgctctgctaatcctgttaccagtggctgctgccagtggcgataagtcgtgtcttaccgggttggactcaagacgatagttaccggataaggcgcagcggtcgggctgaacggggggttcgtgcacacagcccagcttggagcgaacgacctacaccgaactgagatacctacagcgtgagctatgagaaagcgccacgcttcccgaagggagaaaggcggacaggtatccggtaagcggcagggtcggaacaggagagcgcacgagggagcttccagggggaaacgcctggtatctttatagtcctgtcgggtttcgccacctctgacttgagcgtcgatttttgtgatgctcgtcaggggggcggagcctatggaaaaacgccagcaacgcggcctttttacggttcctggccttttgctggccttttgctcacatgttctttcctgcgttatcccctgattctgtggataaccgtattaccgcctttgagtgagctgataccgctcgccgcagccgaacgaccgagcgcagcgagtcagtgagcgaggaagcggaagagcgcccaatacgcaaaccgcctctccccgcgcgttggccgattcattaatgcag

SEQ ID NO: 4 - DNA, 9720 bp, Artificial Sequence
  pAAV-CB-hBB-F8-X5
aattcccatcatcaataatataccttattttggattgaagccaatatgataatgagggggtggagtttgtgacgtggcgcggggcgtgggaacggggcgggtgacgtagtagtctctagaggtccccagcgaccttgacgggcatctgcccggcatttctgacagctttgtgaactgggtggccgagaaggaatgggagttgccgccagattctgacatggatctgaatctgattgagcaggcacccctgaccgtggccgagaagctgcatcgctggcgtaatagcgaagaggcccgcaccgatcgcccttcccaacagttgcgcagcctgaatggcgaatggaattccagacgattgagcgtcaaaatgtaggtatttccatgagcgtttttcctgttgcaatggctggcggtaatattgttctggatattaccagcaaggccgatagtttgagttcttctactcaggcaagtgatgttattactaatcaaagaagtattgcgacaacggttaatttgcgtgatggacagactcttttactcggtggcctcactgattataaaaacacttctcaggattctggcgtaccgttcctgtctaaaatccctttaatcggcctcctgtttagctcccgctctgattctaacgaggaaagcacgttatacgtgctcgtcaaagcaaccatagtacgcgccctgtagcggcgcattaagcgcggcgggtgtggtggttacgcgcagcgtgaccgctacacttgccagcgccctagcgcccgctcctttcgctttcttcccttcctttctcgccacgttcgccggctttccccgtcaagctctaaatcgggggctccctttagggttccgatttagtgctttacggcacctcgaccccaaaaaacttgattagggtgatggttcacgtagtgggccatcgccctgatagacggtttttcgccctttgacgttggagtccacgttctttaatagtggactcttgttccaaactggaacaacactcaaccctatctcggtctattcttttgatttataagggattttgccgatttcggcctattggttaaaaaatgagctgatttaacaaaaatttaacgcgaattttaacaaaatattaacgtttacaatttaaatatttgcttatacaatcttcctgtttttggggcttttctgattatcaaccggggtacatatgattgacatgctagttttacgattaccgttcatcgcctgcaggggggggggggggggggttggccactccctctctgcgcgctcgctcgctcactgaggccgggcgaccaaaggtcgcccgacgcccgggctttgcccgggcggcctcagtgagcgagcgagcgcgcagagagggagtggccaactccatcactaggggttcctagatctgaattcggtacgtacctctggtcgttacataacttacggtaaatggcccgcctggctgaccgcccaacgaccccgcccattgacgtcaataatgacgtatgttcccatagtaacgccaatagggactttccattgacgtcaatgggtggagtatttacggtaaactgcccacttggcagtacatcaagtgtatcatatgccaagtacgccccctattgacgtcaatgacggtaaatggcccgcctggcattatgcccagtacatgaccttatgggactttcctacttggcagtacatctactcgaggccacgttctgcttcactctccccatctcccccccctccccacccccaattttgtatttatttattttttaattattttgtgcagcgatgggggcggggggggggggggggggggcgcgcgccaggcggggcggggcggggcgaggggcggggcggggcgaggcggagaggtgcggcggcagccaatcagagcggcgcgctccgaaagtttccttttatggcgaggcggcggcggcggcggccctataaaaagcgaagcgcgcggcgggcgggagcgggatcagccaccgcggtggcggcctagagtcgacgaggaactgaaaaaccagaaagttaactggtaagtttagtctttttgtcttttatttcaggtcccggatccggtggtggtgcaaatcaaagaactgctcctcagtggatgttgcctttacttctaggcctgtacggaagtgttacttctgctctaaaagctgcggaattgtacccgcggccgcttttcaaaatgcaaatagagctctccacctgcttctttctgtgccttttgcgattctgctttagtgccaccagaagatactacctgggtgcagtggaactgtcatgggactatatgcaaagtgatctcggtgagctgcctgtggacgcaagatttcctcctagagtgccaaaatcttttccattcaacacctcagtcgtgtacaaaaagactctgtttgtagaattcacggatcaccttttcaacatcgctaagccaaggccaccctggatgggtctgctaggtcctaccatccaggctgaggtttatgatacagtggtcgttacacttaagaacatggcttcccatcctgtcagtcttcatgctgttggtgtatcctactggaaatcttctgagggagctgaatatgatgatcagaccagtcaaagggagaaagaagatgataaagtcttccctggtaaaagccatacatatgtctggcaggtcctgaaagagaatggtccaacagcctctgacccaccatgccttacctactcatatctttctcatgtggacctggtaaaagacttgaattcaggcctcattggagccctactagtatgtagagaagggagtctggccaaggaaaagacacagaccttgcacaaatttatactactttttgctgtatttgatgaagggaaaagttggcactcagaaacaaagaactccttgatgcaggatagggatgctgcatctgctcgggcctggcctaaaatgcacacagtcaatggttatgtaaacaggtctctgccaggtctgattggatgccacaggaaatcagtctattggcatgtgattggaatgggcaccactcctgaagtgcactcaatattcctcgaaggtcacacatttcttgtgaggaaccatcgccaggcgtccttggaaatctcgccaataactttccttactgctcaaacactcttgatggaccttggacagtttctactgttttgtcatatctcttcccaccaacatgatggcatggaagcttatgtcaaagtagacagctgtccagaggaaccccaactacgaatgaaaaataatgaagaagcggaagactatgatgatgatcttactgattctgaaatggatgtggtcaggtttgatgatgacaactctccttcctttatccaaattcgctcagttgccaagaagcatcctaaaacttgggtacattacattgctgctgaagaggaggactgggactatgctcccttagtcctcgcccccgatgacagaagttataaaagtcaatatttgaacaatggccctcagcggattggtaggaagtacaaaaaagtccgatttatggcatacacagatgaaacctttaagactcgtgaagctattcagcatgaatcaggaatcttgggacctttactttatggggaagttggagacacactgttgattatatttaagaatcaagcaagcagaccatataacatctaccctcacggaatcactgatgtccgtcctttgtattcaaggagattaccaaaaggtgtaaaacatttgaaggattttccaattctgccaggagaaatattcaaatataaatggacagtgactgtagaagatgggccaactaaatcagatcctcggtgcctgacccgctattactctagtttcgttaatatggagagagatctagcttcaggactcattggccctctcctcatctgctacaaagaatctgtagatcaaagaggaaaccagataatgtcagacaagaggaatgtcatcctgttttctgtatttgatgagaaccgaagctggtacctcacagagaatatacaacgctttctccccaatccagctggagtgcagcttgaggatccagagttccaagcctccaacatcatgcacagcatcaatggctatgtttttgatagtttgcagttgtcagtttgtttgcatgaggtggcatactggtacattctaagcattggagcacagactgacttcctttctgtcttcttctctggatataccttcaaacacaaaatggtctatgaagacacactcaccctattcccattctcaggagaaactgtcttcatgtcgatggaaaacccaggtctatggattctggggtgccacaactcagactttcggaacagaggcatgaccgccttactgaaggtttctagttgtgacaagaacactggtgattattacgaggacagttatgaagatatttcagcatacttgctgagtaaaaacaatgccattgaaccaagaagcttctcccagaattcaagacaccctagcactaggcaaaagcaatttaatgccaccacaccaccagtcttgaaacgccatcaacgcgaaataactcgtactactcttcagtcagatcaagaggaaattgactatgatgataccatatcagttgaaatgaagaaggaagattttgacatttatgatgaggatgaaaatcagagcccccgcagctttcaaaagaaaacacgacactattttattgctgcagtggagaggctctgggattatgggatgagtagctccccacatgttctaagaaacagggctcagagtggcagtgtccctcagttcaagaaagttgttttccaggaatttactgatggctcctttactcagcccttataccgtggagaactaaatgaacatttgggactcctggggccatatataagagcagaagttgaagataatatcatggtaactttcagaaatcaggcctctcgtccctattccttctattctagccttatttcttatgaggaagatcagaggcaaggagcagaacctagaaaaaactttgtcaagcctaatgaaaccaaaacttacttttggaaagtgcaacatcatatggcacccactaaagatgagtttgactgcaaagcctgggcttatttctctgatgttgacctggaaaaagatgtgcactcaggcctgattggaccccttctggtctgccacactaacacactgaaccctgctcatgggagacaagtgacagtacaggaatttgctctgtttttcaccatctttgatgagaccaaaagctggtacttcactgaaaatatggaaagaaactgcagggctccctgcaatatccagatggaagatcccacttttaaagagaattatcgcttccatgcaatcaatggctacataatggatacactacctggcttagtaatggctcaggatcaaaggattcgatggtatctgctcagcatgggcagcaatgaaaacatccattctattcatttcagtggacatgtgttcactgtacgaaaaaaagaggagtataaaatggcactgtacaatctctatccaggtgtttttgagacagtggaaatgttaccatccaaagctggaatttggcgggtggaatgccttattggcgagcatctacatgctgggatgagcacactttttctggtgtacagcaataagtgtcagactcccctgggaatggcttctggacacattagagattttcagattacagcttcaggacaatatggacagtgggccccaaagctggccagacttcattattccggatcaatcaatgcctggagcaccaaggagcccttttcttggatcaaggtggatctgttggcaccaatgattattcacggcatcaagacccagggtgcccgtcagaagttctccagcctctacatctctcagtttatcatcatgtatagtcttgatgggaagaagtggcagacttatcgaggaaattccactggaaccttaatggtcttctttggcaatgtggattcatctgggataaaacacaatatttttaaccctccaattattgctcgatacatccgtttgcacccaactcattatagcattcgcagcactcttcgcatggagttgatgggctgtgatttaaatagttgcagcatgccattgggaatggagagtaaagcaatatcagatgcacagattactgcttcatcctactttaccaatatgtttgccacctggtctccttcaaaagctcgacttcacctccaagggaggagtaatgcctggagacctcaggtgaataatccaaaagagtggctgcaagtggacttccagaagacaatgaaagtcacaggagtaactactcagggagtaaaatctctgcttaccagcatgtatgtgaaggagttcctcatctccagcagtcaagatggccatcagtggactctcttttttcagaatggcaaagtaaaggtttttcagggaaatcaagactccttcacacctgtggtgaactctctagacccaccgttactgactcgctaccttcgaattcacccccagagttgggtgcaccagattgccctgaggatggaggttctgggctgcgaggcacaggacctctactgacaattgacgctgatcagcctcgactgtgccttctagttgccagccatctgttgtttgcccctcccccgtgccttccttgaccctggaaggtgccactcccactgtcctttcctaataaaatgaggaaattgcatcgcattgtctgagtaggtgtcattctattctggggggtggggtggggcaggacagcaagggggaggattgggaagacaatagcaggcatgctggggagagatctaggaacccctagtgatggagttggccactccctctctgcgcgctcgctcgctcactgaggccgcccgggcaaagcccgggcgtcgggcgacctttggtcgcccggcctcagtgagcgagcgagcgcgcagagagggagtggccaacccccccccccccccccctgcaggcgattctcttgtttgctccagactctcaggcaatgacctgatagcctttgtagagacctctcaaaaatagctaccctctccggcatgaatttatcagctagaacggttgaatatcatattgatggtgatttgactgtctccggcctttctcacccgtttgaatctttacctacacattactcaggcattgcatttaaaatatatgagggttctaaaaatttttatccttgcgttgaaataaaggcttctcccgcaaaagtattacagggtcataatgtttttggtacaaccgatttagctttatgctctgaggctttattgcttaattttgctaattctttgccttgcctgtatgatttattggatgttggaattcctgatgcggtattttctccttacgcatctgtgcggtatttcacaccgcatatggtgcactctcagtacaatctgctctgatgccgcatagttaagccagccccgacacccgccaacacccgctgacgcgccctgacgggcttgtctgctcccggcatccgcttacagacaagctgtgaccgtctccgggagctgcatgtgtcagaggttttcaccgtcatcaccgaaacgcgcgagacgaaagggcctcgtgatacgcctatttttataggttaatgtcatgataataatggtttcttagacgtcaggtggcacttttcggggaaatgtgcgcggaacccctatttgtttatttttctaaatacattcaaatatgtatccgctcatgagacaataaccctgataaatgcttcaataatattgaaaaaggaagagtatgagtattcaacatttccgtgtcgcccttattcccttttttgcggcattttgccttcctgtttttgctcacccagaaacgctggtgaaagtaaaagatgctgaagatcagttgggtgcacgagtgggttacatcgaactggatctcaacagcggtaagatccttgagagttttcgccccgaagaacgttttccaatgatgagcacttttaaagttctgctatgtggcgcggtattatcccgtattgacgccgggcaagagcaactcggtcgccgcatacactattctcagaatgacttggttgagtactcaccagtcacagaaaagcatcttacggatggcatgacagtaagagaattatgcagtgctgccataaccatgagtgataacactgcggccaacttacttctgacaacgatcggaggaccgaaggagctaaccgcttttttgcacaacatgggggatcatgtaactcgccttgatcgttgggaaccggagctgaatgaagccataccaaacgacgagcgtgacaccacgatgcctgtagcaatggcaacaacgttgcgcaaactattaactggcgaactacttactctagcttcccggcaacaattaatagactggatggaggcggataaagttgcaggaccacttctgcgctcggcccttccggctggctggtttattgctgataaatctggagccggtgagcgtgggtctcgcggtatcattgcagcactggggccagatggtaagccctcccgtatcgtagttatctacacgacggggagtcaggcaactatggatgaacgaaatagacagatcgctgagataggtgcctcactgattaagcattggtaactgtcagaccaagtttactcatatatactttagattgatttaaaacttcatttttaatttaaaaggatctaggtgaagatcctttttgataatctcatgaccaaaatcccttaacgtgagttttcgttccactgagcgtcagaccccgtagaaaagatcaaaggatcttcttgagatcctttttttctgcgcgtaatctgctgcttgcaaacaaaaaaaccaccgctaccagcggtggtttgtttgccggatcaagagctaccaactctttttccgaaggtaactggcttcagcagagcgcagataccaaatactgtccttctagtgtagccgtagttaggccaccacttcaagaactctgtagcaccgcctacatacctcgctctgctaatcctgttaccagtggctgctgccagtggcgataagtcgtgtcttaccgggttggactcaagacgatagttaccggataaggcgcagcggtcgggctgaacggggggttcgtgcacacagcccagcttggagcgaacgacctacaccgaactgagatacctacagcgtgagctatgagaaagcgccacgcttcccgaagggagaaaggcggacaggtatccggtaagcggcagggtcggaacaggagagcgcacgagggagcttccagggggaaacgcctggtatctttatagtcctgtcgggtttcgccacctctgacttgagcgtcgatttttgtgatgctcgtcaggggggcggagcctatggaaaaacgccagcaacgcggcctttttacggttcctggccttttgctggccttttgctcacatgttctttcctgcgttatcccctgattctgtggataaccgtattaccgcctttgagtgagctgataccgctcgccgcagccgaacgaccgagcgcagcgagtcagtgagcgaggaagcggaagagcgcccaatacgcaaaccgcctctccccgcgcgttggccgattcattaatgcag

SEQ ID NO: 5 - DNA, 7757 bp, Artificial Sequence
  pAAV-CB-hHC1690-X10
aattcccatcatcaataatataccttattttggattgaagccaatatgataatgagggggtggagtttgtgacgtggcgcggggcgtgggaacggggcgggtgacgtagtagtctctagaggtccccagcgaccttgacgggcatctgcccggcatttctgacagctttgtgaactgggtggccgagaaggaatgggagttgccgccagattctgacatggatctgaatctgattgagcaggcacccctgaccgtggccgagaagctgcatcgctggcgtaatagcgaagaggcccgcaccgatcgcccttcccaacagttgcgcagcctgaatggcgaatggaattccagacgattgagcgtcaaaatgtaggtatttccatgagcgtttttcctgttgcaatggctggcggtaatattgttctggatattaccagcaaggccgatagtttgagttcttctactcaggcaagtgatgttattactaatcaaagaagtattgcgacaacggttaatttgcgtgatggacagactcttttactcggtggcctcactgattataaaaacacttctcaggattctggcgtaccgttcctgtctaaaatccctttaatcggcctcctgtttagctcccgctctgattctaacgaggaaagcacgttatacgtgctcgtcaaagcaaccatagtacgcgccctgtagcggcgcattaagcgcggcgggtgtggtggttacgcgcagcgtgaccgctacacttgccagcgccctagcgcccgctcctttcgctttcttcccttcctttctcgccacgttcgccggctttccccgtcaagctctaaatcgggggctccctttagggttccgatttagtgctttacggcacctcgaccccaaaaaacttgattagggtgatggttcacgtagtgggccatcgccctgatagacggtttttcgccctttgacgttggagtccacgttctttaatagtggactcttgttccaaactggaacaacactcaaccctatctcggtctattcttttgatttataagggattttgccgatttcggcctattggttaaaaaatgagctgatttaacaaaaatttaacgcgaattttaacaaaatattaacgtttacaatttaaatatttgcttatacaatcttcctgtttttggggcttttctgattatcaaccggggtacatatgattgacatgctagttttacgattaccgttcatcgcctgcaggggggggggggggggggttggccactccctctctgcgcgctcgctcgctcactgaggccgggcgaccaaaggtcgcccgacgcccgggctttgcccgggcggcctcagtgagcgagcgagcgcgcagagagggagtggccaactccatcactaggggttcctagatctgaattcggtacgtacctctggtcgttacataacttacggtaaatggcccgcctggctgaccgcccaacgaccccgcccattgacgtcaataatgacgtatgttcccatagtaacgccaatagggactttccattgacgtcaatgggtggagtatttacggtaaactgcccacttggcagtacatcaagtgtatcatatgccaagtacgccccctattgacgtcaatgacggtaaatggcccgcctggcattatgcccagtacatgaccttatgggactttcctacttggcagtacatctactcgaggccacgttctgcttcactctccccatctcccccccctccccacccccaattttgtatttatttattttttaattattttgtgcagcgatgggggcggggggggggggggggggggcgcgcgccaggcggggcggggcggggcgaggggcggggcggggcgaggcggagaggtgcggcggcagccaatcagagcggcgcgctccgaaagtttccttttatggcgaggcggcggcggcggcggccctataaaaagcgaagcgcgcggcgggcgggagcgggatcagccaccgcggtggcggcctagagtcgacgaggaactgaaaaaccagaaagttaactggtaagtttagtctttttgtcttttatttcaggtcccggatccggtggtggtgcaaatcaaagaactgctcctcagtggatgttgcctttacttctaggcctgtacggaagtgttacttctgctctaaaagctgcggaattgtacccgcggccgcttttcaaaatgcaaatagagctctccacctgcttctttctgtgccttttgcgattctgctttagtgccaccagaagatactacctgggtgcagtggaactgtcatgggactatatgcaaagtgatctcggtgagctgcctgtggacgcaagatttcctcctagagtgccaaaatcttttccattcaacacctcagtcgtgtacaaaaagactctgtttgtagaattcacggatcaccttttcaacatcgctaagccaaggccaccctggatgggtctgctaggtcctaccatccaggctgaggtttacgacacggtggtcgttaccctgaagaacatggcttctcatcccgttagtcttcacgctgtcggcgtctccttctggaaatcttccgaaggcgctgaatatgaggatcacaccagccaaagggagaaggaagacgataaagtccttcccggtaaaagccaaacctacgtctggcaggtcctgaaagaaaatggtccaacagcctctgacccaccatgtcttacctactcatacctgtctcacgtggacctggtgaaagacctgaattcgggcctcattggagccctactagtatgtagagaagggagtctggccaaggaaaagacacagaccttgcacaaatttatactactttttgctgtatttgatgaagggaaaagttggcactcagaaacaaagaactccttgatgcaggatagggatgctgcatctgctcgggcctggcctaaaatgcacacagtcaatggttatgtaaacaggtctctgccaggtctgattggatgccacaggaaatcagtctattggcatgtgattggaatgggcaccactcctgaagtgcactcaatattcctcgaaggtcacacatttcttgtgaggaaccatcgccaggcgtccttggaaatctcgccaataactttccttactgctcaaacactcttgatggaccttggacagtttctactgttttgtcatatctcttcccaccaacatgatggcatggaagcttatgtcaaagtagacagctgtccagaggaaccccaactacgaatgaaaaataatgaagaagcggaagactatgatgatgatcttactgattctgaaatggatgtggtcaggtttgatgatgacaactctccttcctttatccaaattcgctcagttgccaagaagcatcctaaaacttgggtacattacattgctgctgaagaggaggactgggactatgctcccttagtcctcgcccccgatgacagaagttataaaagtcaatatttgaacaatggccctcagcggattggtaggaagtacaaaaaagtccgatttatggcatacacagatgaaacctttaagactcgtgaagctattcagcatgaatcaggaatcttgggacctttactttatggggaagttggagacacactgttgattatatttaagaatcaagcaagcagaccatataacatctaccctcacggaatcactgatgtccgtcctttgtattcaaggagattaccaaaaggtgtaaaacatttgaaggattttccaattctgccaggagaaatattcaaatataaatggacagtgactgtagaagatgggccaactaaatcagatcctcggtgcctgacccgctattactctagtttcgttaatatggagagagatctagcttcaggactcattggccctctcctcatctgctacaaagaatctgtagatcaaagaggaaaccagataatgtcagacaagaggaatgtcatcctgttttctgtatttgatgagaaccgaagctggtacctcacagagaatatacaacgctttctccccaatccagctggagtgcagcttgaggatccagagttccaagcctccaacatcatgcacagcatcaatggctatgtttttgatagtttgcagttgtcagtttgtttgcatgaggtggcatactggtacattctaagcattggagcacagactgacttcctttctgtcttcttctctggatataccttcaaacacaaaatggtctatgaagacacactcaccctattcccattctcaggagaaactgtcttcatgtcgatggaaaacccaggtctatggattctggggtgccacaactcagactttcggaacagaggcatgaccgccttactgaaggtttctagttgtgacaagaacactggtgattattacgaggacagttatgaagatatttcagcatacttgctgagtaaaaacaatgccattgaaccaagaagcttctcccagaatccaccagtcttgaaacgccatcaacgcgaaataactcgtactactcttcagtcagatcaagaggaaattgactatgatgataccatatcagttgaaatgaagaaggaagattttgacatttatgatgaggatgaaaatcagagcccccgcagctagcaattgtagtctgaacgctgatcagcctcgactgtgccttctagttgccagccatctgttgtttgcccctcccccgtgccttccttgaccctggaaggtgccactcccactgtcctttcctaataaaatgaggaaattgcatcgcattgtctgagtaggtgtcattctattctggggggtggggtggggcaggacagcaagggggaggattgggaagacaatagcaggcatgctggggagagatctaggaacccctagtgatggagttggccactccctctctgcgcgctcgctcgctcactgaggccgcccgggcaaagcccgggcgtcgggcgacctttggtcgcccggcctcagtgagcgagcgagcgcgcagagagggagtggccaacccccccccccccccccctgcaggcgattctcttgtttgctccagactctcaggcaatgacctgatagcctttgtagagacctctcaaaaatagctaccctctccggcatgaatttatcagctagaacggttgaatatcatattgatggtgatttgactgtctccggcctttctcacccgtttgaatctttacctacacattactcaggcattgcatttaaaatatatgagggttctaaaaatttttatccttgcgttgaaataaaggcttctcccgcaaaagtattacagggtcataatgtttttggtacaaccgatttagctttatgctctgaggctttattgcttaattttgctaattctttgccttgcctgtatgatttattggatgttggaattcctgatgcggtattttctccttacgcatctgtgcggtatttcacaccgcatatggtgcactctcagtacaatctgctctgatgccgcatagttaagccagccccgacacccgccaacacccgctgacgcgccctgacgggcttgtctgctcccggcatccgcttacagacaagctgtgaccgtctccgggagctgcatgtgtcagaggttttcaccgtcatcaccgaaacgcgcgagacgaaagggcctcgtgatacgcctatttttataggttaatgtcatgataataatggtttcttagacgtcaggtggcacttttcggggaaatgtgcgcggaacccctatttgtttatttttctaaatacattcaaatatgtatccgctcatgagacaataaccctgataaatgcttcaataatattgaaaaaggaagagtatgagtattcaacatttccgtgtcgcccttattcccttttttgcggcattttgccttcctgtttttgctcacccagaaacgctggtgaaagtaaaagatgctgaagatcagttgggtgcacgagtgggttacatcgaactggatctcaacagcggtaagatccttgagagttttcgccccgaagaacgttttccaatgatgagcacttttaaagttctgctatgtggcgcggtattatcccgtattgacgccgggcaagagcaactcggtcgccgcatacactattctcagaatgacttggttgagtactcaccagtcacagaaaagcatcttacggatggcatgacagtaagagaattatgcagtgctgccataaccatgagtgataacactgcggccaacttacttctgacaacgatcggaggaccgaaggagctaaccgcttttttgcacaacatgggggatcatgtaactcgccttgatcgttgggaaccggagctgaatgaagccataccaaacgacgagcgtgacaccacgatgcctgtagcaatggcaacaacgttgcgcaaactattaactggcgaactacttactctagcttcccggcaacaattaatagactggatggaggcggataaagttgcaggaccacttctgcgctcggcccttccggctggctggtttattgctgataaatctggagccggtgagcgtgggtctcgcggtatcattgcagcactggggccagatggtaagccctcccgtatcgtagttatctacacgacggggagtcaggcaactatggatgaacgaaatagacagatcgctgagataggtgcctcactgattaagcattggtaactgtcagaccaagtttactcatatatactttagattgatttaaaacttcatttttaatttaaaaggatctaggtgaagatcctttttgataatctcatgaccaaaatcccttaacgtgagttttcgttccactgagcgtcagaccccgtagaaaagatcaaaggatcttcttgagatcctttttttctgcgcgtaatctgctgcttgcaaacaaaaaaaccaccgctaccagcggtggtttgtttgccggatcaagagctaccaactctttttccgaaggtaactggcttcagcagagcgcagataccaaatactgtccttctagtgtagccgtagttaggccaccacttcaagaactctgtagcaccgcctacatacctcgctctgctaatcctgttaccagtggctgctgccagtggcgataagtcgtgtcttaccgggttggactcaagacgatagttaccggataaggcgcagcggtcgggctgaacggggggttcgtgcacacagcccagcttggagcgaacgacctacaccgaactgagatacctacagcgtgagctatgagaaagcgccacgcttcccgaagggagaaaggcggacaggtatccggtaagcggcagggtcggaacaggagagcgcacgagggagcttccagggggaaacgcctggtatctttatagtcctgtcgggtttcgccacctctgacttgagcgtcgatttttgtgatgctcgtcaggggggcggagcctatggaaaaacgccagcaacgcggcctttttacggttcctggccttttgctggccttttgctcacatgttctttcctgcgttatcccctgattctgtggataaccgtattaccgcctttgagtgagctgataccgctcgccgcagccgaacgaccgagcgcagcgagtcagtgagcgaggaagcggaagagcgcccaatacgcaaaccgcctctccccgcgcgttggccgattcattaatgcag

SEQ ID NO: 6 - DNA, 7757 bp, Artificial Sequence
  pAAV-CB-hHC1690-X5
aattcccatcatcaataatataccttattttggattgaagccaatatgataatgagggggtggagtttgtgacgtggcgcggggcgtgggaacggggcgggtgacgtagtagtctctagaggtccccagcgaccttgacgggcatctgcccggcatttctgacagctttgtgaactgggtggccgagaaggaatgggagttgccgccagattctgacatggatctgaatctgattgagcaggcacccctgaccgtggccgagaagctgcatcgctggcgtaatagcgaagaggcccgcaccgatcgcccttcccaacagttgcgcagcctgaatggcgaatggaattccagacgattgagcgtcaaaatgtaggtatttccatgagcgtttttcctgttgcaatggctggcggtaatattgttctggatattaccagcaaggccgatagtttgagttcttctactcaggcaagtgatgttattactaatcaaagaagtattgcgacaacggttaatttgcgtgatggacagactcttttactcggtggcctcactgattataaaaacacttctcaggattctggcgtaccgttcctgtctaaaatccctttaatcggcctcctgtttagctcccgctctgattctaacgaggaaagcacgttatacgtgctcgtcaaagcaaccatagtacgcgccctgtagcggcgcattaagcgcggcgggtgtggtggttacgcgcagcgtgaccgctacacttgccagcgccctagcgcccgctcctttcgctttcttcccttcctttctcgccacgttcgccggctttccccgtcaagctctaaatcgggggctccctttagggttccgatttagtgctttacggcacctcgaccccaaaaaacttgattagggtgatggttcacgtagtgggccatcgccctgatagacggtttttcgccctttgacgttggagtccacgttctttaatagtggactcttgttccaaactggaacaacactcaaccctatctcggtctattcttttgatttataagggattttgccgatttcggcctattggttaaaaaatgagctgatttaacaaaaatttaacgcgaattttaacaaaatattaacgtttacaatttaaatatttgcttatacaatcttcctgtttttggggcttttctgattatcaaccggggtacatatgattgacatgctagttttacgattaccgttcatcgcctgcaggggggggggggggggggttggccactccctctctgcgcgctcgctcgctcactgaggccgggcgaccaaaggtcgcccgacgcccgggctttgcccgggcggcctcagtgagcgagcgagcgcgcagagagggagtggccaactccatcactaggggttcctagatctgaattcggtacgtacctctggtcgttacataacttacggtaaatggcccgcctggctgaccgcccaacgaccccgcccattgacgtcaataatgacgtatgttcccatagtaacgccaatagggactttccattgacgtcaatgggtggagtatttacggtaaactgcccacttggcagtacatcaagtgtatcatatgccaagtacgccccctattgacgtcaatgacggtaaatggcccgcctggcattatgcccagtacatgaccttatgggactttcctacttggcagtacatctactcgaggccacgttctgcttcactctccccatctcccccccctccccacccccaattttgtatttatttattttttaattattttgtgcagcgatgggggcggggggggggggggggggggcgcgcgccaggcggggcggggcggggcgaggggcggggcggggcgaggcggagaggtgcggcggcagccaatcagagcggcgcgctccgaaagtttccttttatggcgaggcggcggcggcggcggccctataaaaagcgaagcgcgcggcgggcgggagcgggatcagccaccgcggtggcggcctagagtcgacgaggaactgaaaaaccagaaagttaactggtaagtttagtctttttgtcttttatttcaggtcccggatccggtggtggtgcaaatcaaagaactgctcctcagtggatgttgcctttacttctaggcctgtacggaagtgttacttctgctctaaaagctgcggaattgtacccgcggccgcttttcaaaatgcaaatagagctctccacctgcttctttctgtgccttttgcgattctgctttagtgccaccagaagatactacctgggtgcagtggaactgtcatgggactatatgcaaagtgatctcggtgagctgcctgtggacgcaagatttcctcctagagtgccaaaatcttttccattcaacacctcagtcgtgtacaaaaagactctgtttgtagaattcacggatcaccttttcaacatcgctaagccaaggccaccctggatgggtctgctaggtcctaccatccaggctgaggtttatgatacagtggtcgttacacttaagaacatggcttcccatcctgtcagtcttcatgctgttggtgtatcctactggaaatcttctgagggagctgaatatgatgatcagaccagtcaaagggagaaagaagatgataaagtcttccctggtaaaagccatacatatgtctggcaggtcctgaaagagaatggtccaacagcctctgacccaccatgccttacctactcatatctttctcatgtggacctggtaaaagacttgaattcaggcctcattggagccctactagtatgtagagaagggagtctggccaaggaaaagacacagaccttgcacaaatttatactactttttgctgtatttgatgaagggaaaagttggcactcagaaacaaagaactccttgatgcaggatagggatgctgcatctgctcgggcctggcctaaaatgcacacagtcaatggttatgtaaacaggtctctgccaggtctgattggatgccacaggaaatcagtctattggcatgtgattggaatgggcaccactcctgaagtgcactcaatattcctcgaaggtcacacatttcttgtgaggaaccatcgccaggcgtccttggaaatctcgccaataactttccttactgctcaaacactcttgatggaccttggacagtttctactgttttgtcatatctcttcccaccaacatgatggcatggaagcttatgtcaaagtagacagctgtccagaggaaccccaactacgaatgaaaaataatgaagaagcggaagactatgatgatgatcttactgattctgaaatggatgtggtcaggtttgatgatgacaactctccttcctttatccaaattcgctcagttgccaagaagcatcctaaaacttgggtacattacattgctgctgaagaggaggactgggactatgctcccttagtcctcgcccccgatgacagaagttataaaagtcaatatttgaacaatggccctcagcggattggtaggaagtacaaaaaagtccgatttatggcatacacagatgaaacctttaagactcgtgaagctattcagcatgaatcaggaatcttgggacctttactttatggggaagttggagacacactgttgattatatttaagaatcaagcaagcagaccatataacatctaccctcacggaatcactgatgtccgtcctttgtattcaaggagattaccaaaaggtgtaaaacatttgaaggattttccaattctgccaggagaaatattcaaatataaatggacagtgactgtagaagatgggccaactaaatcagatcctcggtgcctgacccgctattactctagtttcgttaatatggagagagatctagcttcaggactcattggccctctcctcatctgctacaaagaatctgtagatcaaagaggaaaccagataatgtcagacaagaggaatgtcatcctgttttctgtatttgatgagaaccgaagctggtacctcacagagaatatacaacgctttctccccaatccagctggagtgcagcttgaggatccagagttccaagcctccaacatcatgcacagcatcaatggctatgtttttgatagtttgcagttgtcagtttgtttgcatgaggtggcatactggtacattctaagcattggagcacagactgacttcctttctgtcttcttctctggatataccttcaaacacaaaatggtctatgaagacacactcaccctattcccattctcaggagaaactgtcttcatgtcgatggaaaacccaggtctatggattctggggtgccacaactcagactttcggaacagaggcatgaccgccttactgaaggtttctagttgtgacaagaacactggtgattattacgaggacagttatgaagatatttcagcatacttgctgagtaaaaacaatgccattgaaccaagaagcttctcccagaatccaccagtcttgaaacgccatcaacgcgaaataactcgtactactcttcagtcagatcaagaggaaattgactatgatgataccatatcagttgaaatgaagaaggaagattttgacatttatgatgaggatgaaaatcagagcccccgcagctagcaattgtagtctgaacgctgatcagcctcgactgtgccttctagttgccagccatctgttgtttgcccctcccccgtgccttccttgaccctggaaggtgccactcccactgtcctttcctaataaaatgaggaaattgcatcgcattgtctgagtaggtgtcattctattctggggggtggggtggggcaggacagcaagggggaggattgggaagacaatagcaggcatgctggggagagatctaggaacccctagtgatggagttggccactccctctctgcgcgctcgctcgctcactgaggccgcccgggcaaagcccgggcgtcgggcgacctttggtcgcccggcctcagtgagcgagcgagcgcgcagagagggagtggccaacccccccccccccccccctgcaggcgattctcttgtttgctccagactctcaggcaatgacctgatagcctttgtagagacctctcaaaaatagctaccctctccggcatgaatttatcagctagaacggttgaatatcatattgatggtgatttgactgtctccggcctttctcacccgtttgaatctttacctacacattactcaggcattgcatttaaaatatatgagggttctaaaaatttttatccttgcgttgaaataaaggcttctcccgcaaaagtattacagggtcataatgtttttggtacaaccgatttagctttatgctctgaggctttattgcttaattttgctaattctttgccttgcctgtatgatttattggatgttggaattcctgatgcggtattttctccttacgcatctgtgcggtatttcacaccgcatatggtgcactctcagtacaatctgctctgatgccgcatagttaagccagccccgacacccgccaacacccgctgacgcgccctgacgggcttgtctgctcccggcatccgcttacagacaagctgtgaccgtctccgggagctgcatgtgtcagaggttttcaccgtcatcaccgaaacgcgcgagacgaaagggcctcgtgatacgcctatttttataggttaatgtcatgataataatggtttcttagacgtcaggtggcacttttcggggaaatgtgcgcggaacccctatttgtttatttttctaaatacattcaaatatgtatccgctcatgagacaataaccctgataaatgcttcaataatattgaaaaaggaagagtatgagtattcaacatttccgtgtcgcccttattcccttttttgcggcattttgccttcctgtttttgctcacccagaaacgctggtgaaagtaaaagatgctgaagatcagttgggtgcacgagtgggttacatcgaactggatctcaacagcggtaagatccttgagagttttcgccccgaagaacgttttccaatgatgagcacttttaaagttctgctatgtggcgcggtattatcccgtattgacgccgggcaagagcaactcggtcgccgcatacactattctcagaatgacttggttgagtactcaccagtcacagaaaagcatcttacggatggcatgacagtaagagaattatgcagtgctgccataaccatgagtgataacactgcggccaacttacttctgacaacgatcggaggaccgaaggagctaaccgcttttttgcacaacatgggggatcatgtaactcgccttgatcgttgggaaccggagctgaatgaagccataccaaacgacgagcgtgacaccacgatgcctgtagcaatggcaacaacgttgcgcaaactattaactggcgaactacttactctagcttcccggcaacaattaatagactggatggaggcggataaagttgcaggaccacttctgcgctcggcccttccggctggctggtttattgctgataaatctggagccggtgagcgtgggtctcgcggtatcattgcagcactggggccagatggtaagccctcccgtatcgtagttatctacacgacggggagtcaggcaactatggatgaacgaaatagacagatcgctgagataggtgcctcactgattaagcattggtaactgtcagaccaagtttactcatatatactttagattgatttaaaacttcatttttaatttaaaaggatctaggtgaagatcctttttgataatctcatgaccaaaatcccttaacgtgagttttcgttccactgagcgtcagaccccgtagaaaagatcaaaggatcttcttgagatcctttttttctgcgcgtaatctgctgcttgcaaacaaaaaaaccaccgctaccagcggtggtttgtttgccggatcaagagctaccaactctttttccgaaggtaactggcttcagcagagcgcagataccaaatactgtccttctagtgtagccgtagttaggccaccacttcaagaactctgtagcaccgcctacatacctcgctctgctaatcctgttaccagtggctgctgccagtggcgataagtcgtgtcttaccgggttggactcaagacgatagttaccggataaggcgcagcggtcgggctgaacggggggttcgtgcacacagcccagcttggagcgaacgacctacaccgaactgagatacctacagcgtgagctatgagaaagcgccacgcttcccgaagggagaaaggcggacaggtatccggtaagcggcagggtcggaacaggagagcgcacgagggagcttccagggggaaacgcctggtatctttatagtcctgtcgggtttcgccacctctgacttgagcgtcgatttttgtgatgctcgtcaggggggcggagcctatggaaaaacgccagcaacgcggcctttttacggttcctggccttttgctggccttttgctcacatgttctttcctgcgttatcccctgattctgtggataaccgtattaccgcctttgagtgagctgataccgctcgccgcagccgaacgaccgagcgcagcgagtcagtgagcgaggaagcggaagagcgcccaatacgcaaaccgcctctccccgcgcgttggccgattcattaatgcag

SEQ ID NO: 7 - protein, 200 aa, Homo sapiens
ATRRYYLGAVELSWDYMQSDLGELPVDARFPPRVPKSFPFNTSVVYKKTLFVEFTDHLFNIAKPRPPWMGLLGPTIQAEVYDTVVITLKNMASHPVSLHAVGVSYWKASEGAEYDDQTSQREKEDDKVFPGGSHTYVWQVLKENGPMASDPLCLTYSYLSHVDLVKDLNSGLIGALLVCREGSLAKEKTQTLHKFILLFA

SEQ ID NO: 8 - protein, 200 aa, Homo sapiens
ATRRYYLGAVELSWDYMQSDLGELPVDARFPPRVPKSFPFNTSVVYKKTLFVEFTDHLFNIAKPRPPWMGLLGPTIQAEVYDTVVVTLKNMASHPVSLHAVGVSFWKSSEGAEYEDHTSQREKEDDKVLPGKSQTYVWQVLKENGPTASDPPCLTYSYLSHVDLVKDLNSGLIGALLVCREGSLAKEKTQTLHKFILLFA

SEQ ID NO: 9 - protein, 200 aa, Homo sapiens
ATRRYYLGAVELSWDYMQSDLGELPVDARFPPRVPKSFPFNTSVVYKKTLFVEFTDHLFNIAKPRPPWMGLLGPTIQAEVYDTVVVTLKNMASHPVSLHAVGVSYWKSSEGAEYDDQTSQREKEDDKVFPGKSHTYVWQVLKENGPTASDPPCLTYSYLSHVDLVKDLNSGLIGALLVCREGSLAKEKTQTLHKFILLFA